European Patent Application EP 4 722 249 A1, published April 8, 2026. Title: Anti-CD200R1 Antibody and Use Thereof. Applicant: AIMED BIO INC. Application KR. The sequence listing filed with the application follows.

SEQUENCE LISTING (207 sequences)

SEQ ID NO: 1 - protein, 5 aa, synthetic construct
SYDMH

SEQ ID NO: 2 - protein, 5 aa, synthetic construct
SYAMS

SEQ ID NO: 3 - protein, 5 aa, synthetic construct
DYAMS

SEQ ID NO: 4 - protein, 5 aa, synthetic construct
DYYMS

SEQ ID NO: 5 - protein, 5 aa, synthetic construct
GYDMS

SEQ ID NO: 6 - protein, 5 aa, synthetic construct
NYDMS

SEQ ID NO: 7 - protein, 5 aa, synthetic construct
SYDMS

SEQ ID NO: 8 - protein, 5 aa, synthetic construct
NYAMS

SEQ ID NO: 9 - protein, 16 aa, synthetic construct
RISFTGSTSYNPSLKS

SEQ ID NO: 10 - protein, 17 aa, synthetic construct
WISYDSSSKYYADSVKG

SEQ ID NO: 11 - protein, 17 aa, synthetic construct
AISHGGSSKYYADSVKG

SEQ ID NO: 12 - protein, 17 aa, synthetic construct
GIYPGDGSIYYADSVKG

SEQ ID NO: 13 - protein, 17 aa, synthetic construct
QIYPGNGSKYYADSVKG

SEQ ID NO: 14 - protein, 17 aa, synthetic construct
GISYGNGNTYYADSVKG

SEQ ID NO: 15 - protein, 17 aa, synthetic construct
AISYDNGNTYYADSVKG

SEQ ID NO: 16 - protein, 17 aa, synthetic construct
WISHGGGSIYYADSVKG

SEQ ID NO: 17 - protein, 17 aa, synthetic construct
SISPGGGSIYYADSVKG

SEQ ID NO: 18 - protein, 17 aa, synthetic construct
WISSGGGSTYYADSVKG

SEQ ID NO: 19 - protein, 17 aa, synthetic construct
GISSSGGNKYYADSVKG

SEQ ID NO: 20 - protein, 17 aa, synthetic construct
GIPPGDGSTYYADSVKG

SEQ ID NO: 21 - protein, 17 aa, synthetic construct
GISYDGGSKYYADSVKG

SEQ ID NO: 22 - protein, 10 aa, synthetic construct
DTWWEGYFDL

SEQ ID NO: 23 - protein, 13 aa, synthetic construct
GVVQPYLWTEFDY

SEQ ID NO: 24 - protein, 10 aa, synthetic construct
GPEVMLEFDY

SEQ ID NO: 25 - protein, 12 aa, synthetic construct
GLDLYEPMAFDY

SEQ ID NO: 26 - protein, 12 aa, synthetic construct
DLQTWTSRRFDY

SEQ ID NO: 27 - protein, 12 aa, synthetic construct
DPWQTAINDFDY

SEQ ID NO: 28 - protein, 7 aa, synthetic construct
NRAWFDY

SEQ ID NO: 29 - protein, 12 aa, synthetic construct
DAPALMHSLFDY

SEQ ID NO: 30 - protein, 12 aa, synthetic construct
DAPAYSAPLFDY

SEQ ID NO: 31 - protein, 12 aa, synthetic construct
DPGQMFWPLFDY

SEQ ID NO: 32 - protein, 18 aa, synthetic construct
VRGTCNGTLCYYSNAMDV

SEQ ID NO: 33 - protein, 18 aa, synthetic construct
AIRPCISAPCYYDDAMDV

SEQ ID NO: 34 - protein, 18 aa, synthetic construct
HLVSDHPPSQYSDDGMDV

SEQ ID NO: 35 - protein, 12 aa, synthetic construct
DGYPLGAYYFDY

SEQ ID NO: 36 - protein, 13 aa, synthetic construct
SGSSSNIGNNHVS

SEQ ID NO: 37 - protein, 13 aa, synthetic construct
SGSSSNIGSNYVN

SEQ ID NO: 38 - protein, 13 aa, synthetic construct
TGSSSNIGNNAVT

SEQ ID NO: 39 - protein, 13 aa, synthetic construct
SGSSSNIGNNDVN

SEQ ID NO: 40 - protein, 13 aa, synthetic construct
TGSSSNIGNNSVN

SEQ ID NO: 41 - protein, 13 aa, synthetic construct
SGSSSNIGNNNVY

SEQ ID NO: 42 - protein, 13 aa, synthetic construct
SGSSSNIGSNHVN

SEQ ID NO: 43 - protein, 13 aa, synthetic construct
SGSSSNIGNNAVN

SEQ ID NO: 44 - protein, 13 aa, synthetic construct
TGSSSNIGSNNVS

SEQ ID NO: 45 - protein, 13 aa, synthetic construct
TGSSSNIGSNDVS

SEQ ID NO: 46 - protein, 13 aa, synthetic construct
TGSSSNIGSNYVS

SEQ ID NO: 47 - protein, 13 aa, synthetic construct
SVSSSNIGSNYVS

SEQ ID NO: 48 - protein, 7 aa, synthetic construct
DTDRLTS

SEQ ID NO: 49 - protein, 7 aa, synthetic construct
SDSHRPS

SEQ ID NO: 50 - protein, 7 aa, synthetic construct
SDNHRPS

SEQ ID NO: 51 - protein, 7 aa, synthetic construct
SNSHRPS

SEQ ID NO: 52 - protein, 7 aa, synthetic construct
TNSHRPS

SEQ ID NO: 53 - protein, 7 aa, synthetic construct
YDSQRPS

SEQ ID NO: 54 - protein, 7 aa, synthetic construct
YDSNRPS

SEQ ID NO: 55 - protein, 7 aa, synthetic construct
DDSHRPS

SEQ ID NO: 56 - protein, 7 aa, synthetic construct
DDNHRPS

SEQ ID NO: 57 - protein, 7 aa, synthetic construct
YNSQRPS

SEQ ID NO: 58 - protein, 7 aa, synthetic construct
DDSKRPS

SEQ ID NO: 59 - protein, 11 aa, synthetic construct
GTWDSSLSAYV

SEQ ID NO: 60 - protein, 11 aa, synthetic construct
GSWDDSLSGYV

SEQ ID NO: 61 - protein, 11 aa, synthetic construct
AAWDSSLSGYV

SEQ ID NO: 62 - protein, 11 aa, synthetic construct
GTWDDSLNGYV

SEQ ID NO: 63 - protein, 11 aa, synthetic construct
GTWDSSLSGYV

SEQ ID NO: 64 - protein, 11 aa, synthetic construct
AAWDASLNGYV

SEQ ID NO: 65 - protein, 11 aa, synthetic construct
GSWDASLNGYV

SEQ ID NO: 66 - protein, 11 aa, synthetic construct
AAWDDSLSGYV

SEQ ID NO: 67 - protein, 11 aa, synthetic construct
GTWDASLNAYV

SEQ ID NO: 68 - protein, 11 aa, synthetic construct
GSWDYSLSAYV

SEQ ID NO: 69 - protein, 11 aa, synthetic construct
GSWDYSLNGYV

SEQ ID NO: 70 - protein, 11 aa, synthetic construct
GTWDASLNGYV

SEQ ID NO: 71 - protein, 118 aa, synthetic construct
EVQLLESGGGLVQPGGSLRLSCAASGFTFSSYDMHWVRQAPGKGLEWVSRISFTGSTSYNPSLKSRFTISRDNSKNTLYLQMNSLRAEDTAVYYCARDTWWEGYFDLWGQGTLVTVSS

SEQ ID NO: 72 - protein, 122 aa, synthetic construct
EVQLLESGGGLVQPGGSLRLSCAASGFTFSSYAMSWVRQAPGKGLEWVSWISYDSSSKYYADSVKGRFTISRDNSKNTLYLQMNSLRAEDTAVYYCARGVVQPYLWTEFDYWGQGTLVTVSS

SEQ ID NO: 73 - protein, 119 aa, synthetic construct
EVQLLESGGGLVQPGGSLRLSCAASGFTFSDYAMSWVRQAPGKGLEWVSAISHGGSSKYYADSVKGRFTISRDNSKNTLYLQMNSLRAEDTAVYYCARGPEVMLEFDYWGQGTLVTVSS

SEQ ID NO: 74 - protein, 121 aa, synthetic construct
EVQLLESGGGLVQPGGSLRLSCAASGFTFSDYYMSWVRQAPGKGLEWVSGIYPGDGSIYYADSVKGRFTISRDNSKNTLYLQMNSLRAEDAAVYYCAKGLDLYEPMAFDYWGQGTLVTVSS

SEQ ID NO: 75 - protein, 121 aa, synthetic construct
EVQLLESGGGLVQPGGSLRLSCAASGFTFSGYDMSWVRQAPGKGLEWVSQIYPGNGSKYYADSVKGRFTISRDNSKNALYLQMNSLRAEDTAVYYCAKDLQTWTSRRFDYWGQGTLVTVSS

SEQ ID NO: 76 - protein, 121 aa, synthetic construct
EVQLLESGGGLVQPGGSLRLSCAASGFTFSDYAMSWVRQAPGKGLEWVSGISYGNGNTYYADSVKGRFTISRDNSKNTLYLQMNSLRAEDTAVYYCAKDPWQTAINDFDYWGQGTLVTVSS

SEQ ID NO: 77 - protein, 116 aa, synthetic construct
EVQLLESGGGLVQPGGSLRLSCAASGFTFSNYDMSWVRQAPGKGLEWVSAISYDNGNTYYADSVKGRFTISRDNSKNTLYLQMNSLRAEDTAVYYCARNRAWFDYWGQGTLVTVSS

SEQ ID NO: 78 - protein, 121 aa, synthetic construct
EVQLLESGGGLVQPGGSLRLSCAASGFTFSSYDMSWVRQAPGKGLEWVSWISHGGGSIYYADSVKGRFTISRDNSKNTLYLQMNSLRAEDTAVYYCARDAPALMHSLFDYWGQGTLVTVSS

SEQ ID NO: 79 - protein, 121 aa, synthetic construct
EVQLLESGGGLVQPGGSLRLSCAASGFTFSSYDMSWVRQAPGKGLEWVSWISHGGGSIYYADSVKGRFTISRDNSKNTLYLQMNSLRAEDTAVYYCARDAPAYSAPLFDYWGQGTLVTVSS

SEQ ID NO: 80 - protein, 121 aa, synthetic construct
EVQLLESGGGLVQPGGSLRLSCAASGFTFSNYAMSWVRQAPGKGLEWVSSISPGGGSIYYADSVKGRFTISRDNSKNTLYLQMNSLRAEDTAVYYCARDPGQMFWPLFDYWGQGTLVTVSS

SEQ ID NO: 81 - protein, 127 aa, synthetic construct
EVQLLESGGGLVQPGGSLRLSCAASGFTFSDYYMSWVRQAPGKGLEWVSWISSGGGSTYYADSVKGRFTISRDNSKNTLYLQMNSLGAEDTAVYYCARVRGTCNGTLCYYSNAMDVWGQGTLVTVSS

SEQ ID NO: 82 - protein, 127 aa, synthetic construct
EVQLLESGGGLVQPGGSLRLSCAASGFTFSGYDMSWVRQAPGKGLEWVSGISSSGGNKYYADSVKGRFTISRDNSKNTLYLQMNSLRAEDTAVYYCARAIRPCISAPCYYDDAMDVWGQGTLVTVSS

SEQ ID NO: 83 - protein, 127 aa, synthetic construct
EVQLLESGGGLVQPGGSLRLSCAASGFTFSGYDMSWVRQAPGKGLEWVSGIPPGDGSTYYADSVKGRFTISRDNSKNTLYLQMNSLRAEDTAVYYCAKHLVSDHPPSQYSDDGMDVWGQGTLVTVSS

SEQ ID NO: 84 - protein, 121 aa, synthetic construct
EVQLLESGGGLVQPGGSLRLSCAASGFTFSSYDMSWVRQVPGKGLEWVSWISHGGGSIYYADSVKGRFTISRDNSKNTLYLQMNSLRAEDTAVYYCARDAPAYSAPLFDYWGQGTLVTVSS

SEQ ID NO: 85 - protein, 121 aa, synthetic construct
EVQLLESGGGLVQPGGSLRLSCAASGFTFSGYDMSWVRQAPGKGLEWVSGISYDGGSKYYADSVKGRFTISRDNSKNTLYLQMNSLRAEDTAVYYCAKDGYPLGAYYFDYWGQGTLVTVSS

SEQ ID NO: 86 - protein, 110 aa, synthetic construct
QSVLTQPPSASGTPGQRVTISCSGSSSNIGNNHVSWYQQLPGTAPKLLIYDDTDRLTSVPNRFSGSKSGTSASLAISGLRSEDEADYYCGTWDSSLSAYVFGGGTKLTVL

SEQ ID NO: 87 - protein, 110 aa, synthetic construct
QSVLTQPPSASGTPGQRVTISCSGSSSNIGSNYVNWYQQLPGTAPKLLIYSDSHRPSGVPDRFSGSKSGTSASLAISGLRSEDEADYYCGSWDDSLSGYVFGGGTKLTVL

SEQ ID NO: 88 - protein, 110 aa, synthetic construct
QSVLTQPPSASGTPGQRVTISCTGSSSNIGNNAVTWYQQLPGTAPKLLIYSDNHRPSGVPDRFSGSKSGTSASLAISGLRSEDEADYYCAAWDSSLSGYVFGGGTKLTVL

SEQ ID NO: 89 - protein, 110 aa, synthetic construct
QSVLTQPPSASGTPGQRVTISCSGSSSNIGSNYVNWYQQLPGTAPKLLIYSNSHRPSGVPDRFSGSKSGTSASLAISGLRSEDGADYYCGTWDDSLNGYVFGGGTKLTVL

SEQ ID NO: 90 - protein, 110 aa, synthetic construct
QSVLTQPPSASGTPGQRVTISCSGSSSNIGNNDVNWYQQLPGTAPKLLIYSNSHRPSGVPDRFSGSKSGTSASLAISGLRSEDGADYYCGTWDDSLNGYVFGGGTKLTVL

SEQ ID NO: 91 - protein, 110 aa, synthetic construct
QSVLTQPPSASGTPGQRVTISCTGSSSNIGNNSVNWYQQLPGTAPKLLIYTNSHRPSEVPDRFSGSKSGTSASLAISGLRSEDEADYYCGTWDSSLSGYVFGGGTKLTVL

SEQ ID NO: 92 - protein, 110 aa, synthetic construct
QSVLTQPPSASGTPGQRVTISCSGSSSNIGNNNVYWYQQLPGTAPKLLIYYDSQRPSGVPDRFSGSKSGTSASLAISGLRSEDEADYYCAAWDASLNGYVFGGGTKLTVL

SEQ ID NO: 93 - protein, 110 aa, synthetic construct
QSVLTQPPSASGTPGQRVTISCSGSSSNIGSNHVNWYQQLPGTAPKLLIYYDSQRPSGVPDRFSGSKSGTSASLAISGLRSEDEADYYCGSWDASLNGYVFGGGTKLTVL

SEQ ID NO: 94 - protein, 110 aa, synthetic construct
QSVLTQPPSASGTPGQRVTISCSGSSSNIGNNAVNWYQQLPGTAPKLLIYYDSNRPSGVPDRFSGSKSGTSASLAISGLRSEDEADYYCAAWDDSLSGYVFGGGTKLTVL

SEQ ID NO: 95 - protein, 110 aa, synthetic construct
QSVLTQPPSASGTPGQRVTISCTGSSSNIGSNNVSWYQQLPGTAPKLLIYDDSHRPSGVPDRFSGSKSGTSASLAISGLRSEDEADYYCGSWDASLNGYVFGGGTKLTVL

SEQ ID NO: 96 - protein, 110 aa, synthetic construct
QSVLTQPPSASGTPGQRVTISCTGSSSNIGSNDVSWYQQLPGTAPKLLIYDDNHRPSGVPDRFSGSKSGTSASLAISGLRSEDEADYYCGTWDASLNAYVFGGGTKLTVL

SEQ ID NO: 97 - protein, 110 aa, synthetic construct
QSVLTQPPSASGTPGQRVTISCTGSSSNIGSNYVSWYRQLPGTAPKLLIYSDSQRPSGVPDRFSGSKSGTSASLAISGLRSEDEADYYCGSWDYSLSAYVFGGGTKLTVL

SEQ ID NO: 98 - protein, 110 aa, synthetic construct
QSVLTQPPSASGTPGQRVTISCSGSSSNIGNNDVNWYQQLPGTAPKLLIYYNSQRPSGVPDRFSGSKSGTSASLAISGLRSEDEADYYCGSWDYSLNGYVFGGGTKLTVL

SEQ ID NO: 99 - protein, 110 aa, synthetic construct
QSVLTQPPSASGTPGQRVTISCSVSSSNIGSNYVSWYRQLPGTAPKLLIYDDSKRPSGVPDRFSGSKSGTSASLAISGLRSEDEADYYCGTWDASLNGYVFGGGTKLTVL

SEQ ID NO: 100 - protein, 5 aa, synthetic construct
SYWMN

SEQ ID NO: 101 - protein, 5 aa, synthetic construct
SYWIN

SEQ ID NO: 102 - protein, 5 aa, synthetic construct
SYWMQ

SEQ ID NO: 103 - protein, 5 aa, synthetic construct
DYYLH

SEQ ID NO: 104 - protein, 17 aa, synthetic construct
RIDPADSEIHYNQKFKD

SEQ ID NO: 105 - protein, 17 aa, synthetic construct
DINPGSGSTNYNEKFRS

SEQ ID NO: 106 - protein, 17 aa, synthetic construct
RIDPSDSETHYNQKFKD

SEQ ID NO: 107 - protein, 17 aa, synthetic construct
AIYPGDGDTRYTQKFKG

SEQ ID NO: 108 - protein, 17 aa, synthetic construct
WIDPENGDTEYAPKFQG

SEQ ID NO: 109 - protein, 17 aa, synthetic construct
RIDPYDSETHYNQKFKD

SEQ ID NO: 110 - protein, 10 aa, synthetic construct
SGGWLPGFAY

SEQ ID NO: 111 - protein, 10 aa, synthetic construct
EDYYGSRFFY

SEQ ID NO: 112 - protein, 10 aa, synthetic construct
SGGWLPGFAY

SEQ ID NO: 113 - protein, 13 aa, synthetic construct
GGVTTLVPYFFDY

SEQ ID NO: 114 - protein, 4 aa, synthetic construct
GGSY

SEQ ID NO: 115 - protein, 9 aa, synthetic construct
VDGNHLFDY

SEQ ID NO: 116 - protein, 10 aa, synthetic construct
SASSSLIYMH

SEQ ID NO: 117 - protein, 16 aa, synthetic construct
RSSQSLVHSNGNTYLH

SEQ ID NO: 118 - protein, 10 aa, synthetic construct
SARSSVSYMH

SEQ ID NO: 119 - protein, 16 aa, synthetic construct
RSSQSIVHSNGNTYLE

SEQ ID NO: 120 - protein, 10 aa, synthetic construct
SASSSLSYML

SEQ ID NO: 121 - protein, 17 aa, synthetic construct
KSSQSLLNSGNQKNYLA

SEQ ID NO: 122 - protein, 11 aa, synthetic construct
KASQDINSYLS

SEQ ID NO: 123 - protein, 7 aa, synthetic construct
DTSKLAS

SEQ ID NO: 124 - protein, 7 aa, synthetic construct
KVSNRFS

SEQ ID NO: 125 - protein, 7 aa, synthetic construct
DTSKLAS

SEQ ID NO: 126 - protein, 7 aa, synthetic construct
GASTRES

SEQ ID NO: 127 - protein, 7 aa, synthetic construct
RANRLVD

SEQ ID NO: 128 - protein, 11 aa, synthetic construct
FQGSGYPLMYT

SEQ ID NO: 129 - protein, 7 aa, synthetic construct
SQSTHVT

SEQ ID NO: 130 - protein, 11 aa, synthetic construct
FQGSGDPLMYT

SEQ ID NO: 131 - protein, 9 aa, synthetic construct
FQGSHVPPT

SEQ ID NO: 132 - protein, 11 aa, synthetic construct
FQGSGNPLMYT

SEQ ID NO: 133 - protein, 9 aa, synthetic construct
QNDHSYPYT

SEQ ID NO: 134 - protein, 9 aa, synthetic construct
LQYDEFPYT

SEQ ID NO: 135 - protein, 119 aa, synthetic construct
QVQLQQPGAEFVKPGAPVKLSCKASGYTFTSYWMNWVKQRPGRGLEWIGRIDPADSEIHYNQKFKDKATLTVDKSSSTAYIQFSSLTSEDSAVYYCARSGGWLPGFAYWGQGTLVTVSA

SEQ ID NO: 136 - protein, 119 aa, synthetic construct
QVQLQQPGAELVKPGTSVKLSCKASGYNFTSYWINWVKLRPGQGLEWIGDINPGSGSTNYNEKFRSKATLTVGTSSSTAYMQLSSLASEDSALYYCAREDYYGSRFFYWGQGTLVTVSA

SEQ ID NO: 137 - protein, 119 aa, synthetic construct
QVQLQQPGAELVKPGAPVKLSCKASGFTLTSYWMNWVKQRPGRGLEWIGRIDPSDSETHYNQKFKDKATLTVDKSSSTAYIQLTSLTSEDSAVYYCARSGGWLPGFAYWGQGTLVTVSA

SEQ ID NO: 138 - protein, 122 aa, synthetic construct
QVQLQQSGAELARPGASVKLSCKASGYTFTSYWMQWVKQRPGQGLEWIGAIYPGDGDTRYTQKFKGKATLTADKSSSTAYMQLRSLASEDSAVFYCARGGVTTLVPYFFDYWGQGATLTVSS

SEQ ID NO: 139 - protein, 119 aa, synthetic construct
QVQLQQPGAELVKPGAPVKLSCKASGYTFTSYWMNWVKQRPGRGLEWIGRIDPSDSETHYNQKFKDKATLTVDKSSSTAYIQLSSLTSEDSAVYYCARSGGWLPGFAYWGQGTLVTVSA

SEQ ID NO: 140 - protein, 111 aa, synthetic construct
QLQQSGAELVRSGASVKLSCTASGFNIKDYYLHWIKQRPEQGLEWIGWIDPENGDTEYAPKFQGKATMTADTSSNTAYLQLISLTSEDAAVYYCFAGGSYWGQGTSVTVSS

SEQ ID NO: 141 - protein, 118 aa, synthetic construct
QVQLQQPGAELVRPGASVKLSCKASAYTFTSYWMNWVKQRPEQGLEWIGRIDPYDSETHYNQKFKDKAILTVDKSSSTAYMQLSSLTSEDSAVYYCARVDGNHLFDYWGQGTTLTVSS

SEQ ID NO: 142 - protein, 108 aa, synthetic construct
ENVLTQSPAIMSASPGEKVTMTCSASSSLIYMHWYQQKSSTSPKLWIYDTSKLASGVPGRFSGSGSGNSYSLTINSMEAEDVATYYCFQGSGYPLMYTFGGGTKLEIK

SEQ ID NO: 143 - protein, 110 aa, synthetic construct
DVVMTQTPLSLPVSLGDQASISCRSSQSLVHSNGNTYLHWYLQKPGQSPKLLIYKVSNRFSGVPDRFSGSGSGTDFTLKISRVEAEDLGVYFCSQSTHVTFGAGTKLELK

SEQ ID NO: 144 - protein, 108 aa, synthetic construct
ENVLTQSPAIMSASPGEKVTMTCSARSSVSYMHWYQQKSRTSPKLWIYDTSKLASGVPGRFSGSGSGNSYSLTISSMEAEDVATYYCFQGSGDPLMYTFGGGTKLEIK

SEQ ID NO: 145 - protein, 112 aa, synthetic construct
DVLMTQTPLSLPVSLGDQASISCRSSQSIVHSNGNTYLEWYLQKPGQSPKLLIYKVSNRFSGVPDRFSGSGSGTDFTLKISRVEAEDLGVYYCFQGSHVPPTFGGGTKLEIK

SEQ ID NO: 146 - protein, 108 aa, synthetic construct
ENVLTQSPAIMSASPGEKVTMTCSASSSLSYMLWYQQKSSTSPKLWIYDTSKLASGVPGRFSGSGSGNSYSLTISSMEAEDVGTYYCFQGSGNPLMYTFGGGTKLEIK

SEQ ID NO: 147 - protein, 113 aa, synthetic construct
DIVMTQSPSSLSVSAGEKVTMSCKSSQSLLNSGNQKNYLAWYQQKPGQPPKLLIYGASTRESGVPDRFTGSGSGTDFTLTISSVQAEDLAVYYCQNDHSYPYTFGGGTKLEIK

SEQ ID NO: 148 - protein, 107 aa, synthetic construct
DIKMTQSPSSMYASLGERVTITCKASQDINSYLSWFQQKPGKSPKTLIYRANRLVDGVPSRFSGSGSGQDYSLTISSLEYEDMGIYYCLQYDEFPYTFGGGTKLEIK

SEQ ID NO: 149 - protein, 119 aa, synthetic construct
EVKLQQSGPELVKPGASVKMSCKASGYTFTSYVMHWVKQKPGQGLEWIGYINPYNDDTNYNEKFKGKATLTSDKSSSTAYMELSSLTSEDSAVYYCAREDYYGSRWGYWGQGTTLTVSS

SEQ ID NO: 150 - protein, 119 aa, synthetic construct
QVQLVQSGAEVKKPGASVKVSCKASGYTFTSYVMHWVRQAPGQGLEWMGYINPYNDDTNYNEKFKGRVTMTRDTSTSTVYMELSSLRSEDTAVYYCAREDYYGSRWGYWGQGTLVTVSS

SEQ ID NO: 151 - protein, 119 aa, synthetic construct
QVQLVQSGAEVKKPGASVKVSCKASGYTFTSYVMHWVRQAPGQGLEWIGYINPYNDDTNYNEKFKGRATLTSDKSTSTAYMELSSLRSEDTAVYYCAREDYYGSRWGYWGQGTLVTVSS

SEQ ID NO: 152 - protein, 119 aa, synthetic construct
QVQLVESGGGVVQPGGSLRLSCAASGYTFTSYVMHWVRQAPGKGLEWVAYINPYNDDTNYNEKFKGRFTISRDNSKNTLYLQMNSLRAEDTAVYYCAKEDYYGSRWGYWGQGTLVTVSS

SEQ ID NO: 153 - protein, 119 aa, synthetic construct
EVQLVESGGGVVQPGGSLRLSCAASGYTFTSYVMHWVRQAPGKGLEWIGYINPYNDDTNYNEKFKGRATLSSDKSKNTAYLQMNSLRAEDTAVYYCAREDYYGSRWGYWGQGTLVTVSS

SEQ ID NO: 154 - protein, 110 aa, synthetic construct
DIVLTQSPASLAVSLGQRATISCRASKSVSTSGYSYMHWYQQKPGQPPKLLIYLASNLESGVPARFSGSGSGTDFTLNIHPVEEEDAATYYCQHSRELLTFGAGTKLELK

SEQ ID NO: 155 - protein, 110 aa, synthetic construct
DIVLTQSPASLAVSPGQRATITCRASKSVSTSGYSYMHWYQQKPGQPPKLLIYLASNLESGVPARFSGSGSGTDFTLTINPVEANDTANYYCQHSRELLTFGQGTKVEIK

SEQ ID NO: 156 - protein, 110 aa, synthetic construct
DIVLTQSPASLAVSPGQRATITCRASKSVSTSGYSYMHWYQQKPGQPPKLLIYLASNLESGVPARFSGSGSGTDFTLTINPVEANDTANYYCQHSRELLTFGAGTKVEIK

SEQ ID NO: 157 - protein, 110 aa, synthetic construct
DIQMTQSPSSLSASVGDRVTITCRASKSVSTSGYSYMHWYQQKPGKAPKLLIYLASNLESGVPSRFSGSGSGTDFTLTISSLQPEDFATYYCQHSRELLTFGQGTKVEIK

SEQ ID NO: 158 - protein, 5 aa, synthetic construct
SYVMH

SEQ ID NO: 159 - protein, 17 aa, synthetic construct
YINPYNDDTNYNEKFKG

SEQ ID NO: 160 - protein, 10 aa, synthetic construct
EDYYGSRWGY

SEQ ID NO: 161 - protein, 15 aa, synthetic construct
RASKSVSTSGYSYMH

SEQ ID NO: 162 - protein, 7 aa, synthetic construct
LASNLES

SEQ ID NO: 163 - protein, 8 aa, synthetic construct
QHSRELLT

SEQ ID NO: 164 - protein, 244 aa, synthetic construct
QVQLVQSGAEVKKPGASVKVSCKASGYTFTSYVMHWVRQAPGQGLEWMGYINPYNDDTNYNEKFKGRVTMTRDTSTSTVYMELSSLRSEDTAVYYCAREDYYGSRWGKWGQGTLVTVSSGGGGSGGGGSGGGGSDIVLTQSPASLAVSPGQRATITCRASKSVSTSGYSYMHWYQQKPGQPPKLLIYLASNLESGVPARFSGSGSGTDFTLTINPVEANDTANYYCQHSRELLTFGQGTKVEIK

SEQ ID NO: 165 - protein, 244 aa, synthetic construct
QVQLVQSGAEVKKPGASVKVSCKASGYTFTSYVMHWVRQAPGQGLEWMGYINPYNDDTNYNEKFKGRVTMTRDTSTSTVYMELSSLRSEDTAVYYCAREDYYGSRWGTWGQGTLVTVSSGGGGSGGGGSGGGGSDIVLTQSPASLAVSPGQRATITCRASKSVSTSGYSYMHWYQQKPGQPPKLLIYLASNLESGVPARFSGSGSGTDFTLTINPVEANDTANYYCQHSRELLTFGQGTKVEIK

SEQ ID NO: 166 - protein, 244 aa, synthetic construct
QVQLVQSGAEVKKPGASVKVSCKASGYTFTSYVMHWVRQAPGQGLEWMGYINPYNDDTNYNEKFKGRVTMTRDTSTSTVYMELSSLRSEDTAVYYCAREDYYGSRWGYWGQGTLVTVSSGGGGSGGGGSGGGGSDIVLTQSPASLAVSPGQRATITCRASKSVSTSGYSYMHWYQQKPGQPPKLLIYLASNLESGVPARFSGSGSGTDFTLTINPVEANDTANYYCQHSHELLTFGQGTKVEIK

SEQ ID NO: 167 - protein, 244 aa, synthetic construct
QVQLVQSGAEVKKPGASVKVSCKASGYTFTSYVMHWVRQAPGQGLEWMGYINPYNDDTNYNEKFKGRVTMTRDTSTSTVYMELSSLRSEDTAVYYCAREDYYGSRWGYWGQGTLVTVSSGGGGSGGGGSGGGGSDIVLTQSPASLAVSPGQRATITCRASKSVSTSGYSYMHWYQQKPGQPPKLLIYLASNLESGVPARFSGSGSGTDFTLTINPVEANDTANYYCQHSSELLTFGQGTKVEIK

SEQ ID NO: 168 - protein, 244 aa, synthetic construct
QVQLVQSGAEVKKPGASVKVSCKASGYTFTSYVMHWVRQAPGQGLEWMGYINPYNDDTNYNEKFKGRVTMTRDTSTSTVYMELSSLRSEDTAVYYCAREDYYGSRWGYWGQGTLVTVSSGGGGSGGGGSGGGGSDIVLTQSPASLAVSPGQRATITCRASKSVSTSGYSYMHWYQQKPGQPPKLLIYLASNLESGVPARFSGSGSGTDFTLTINPVEANDTANYYCQHSRESLTFGQGTKVEIK

SEQ ID NO: 169 - protein, 244 aa, synthetic construct
QVQLVQSGAEVKKPGASVKVSCKASGYTFTSYVMHWVRQAPGQGLEWMGYINPYNDDTNYNEKFKGRVTMTRDTSTSTVYMELSSLRSEDTAVYYCAREDYYGSRWGYWGQGTLVTVSSGGGGSGGGGSGGGGSDIVLTQSPASLAVSPGQRATITCRASKSVSTSGYSYMHWYQQKPGQPPKLLIYLASNLESGVPARFSGSGSGTDFTLTINPVEANDTANYYCQHSREHLTFGQGTKVEIK

SEQ ID NO: 170 - protein, 244 aa, synthetic construct
QVQLVQSGAEVKKPGASVKVSCKASGYTFTSYVMHWVRQAPGQGLEWMGYINPYNDDTNYNEKFKGRVTMTRDTSTSTVYMELSSLRSEDTAVYYCAREDYYGSRWGYWGQGTLVTVSSGGGGSGGGGSGGGGSDIVLTQSPASLAVSPGQRATITCRASKSVSTSGYSYMHWYQQKPGQPPKLLIYLASNLESGVPARFSGSGSGTDFTLTINPVEANDTANYYCQHSRELDTFGQGTKVEIK

SEQ ID NO: 171 - protein, 244 aa, synthetic construct
QVQLVQSGAEVKKPGASVKVSCKASGYTFTSYVMHWVRQAPGQGLEWMGYINPYNDDTNYNEKFKGRVTMTRDTSTSTVYMELSSLRSEDTAVYYCAREDYYGSRWGYWGQGTLVTVSSGGGGSGGGGSGGGGSDIVLTQSPASLAVSPGQRATITCRASKSVSTSGYSYMHWYQQKPGQPPKLLIYLASNLESGVPARFSGSGSGTDFTLTINPVEANDTANYYCQHSRELLRFGQGTKVEIK

SEQ ID NO: 172 - protein, 10 aa, synthetic construct
EDYYGSRWGK

SEQ ID NO: 173 - protein, 10 aa, synthetic construct
EDYYGSRWGT

SEQ ID NO: 174 - protein, 8 aa, synthetic construct
QHSHELLT

SEQ ID NO: 175 - protein, 8 aa, synthetic construct
QHSSELLT

SEQ ID NO: 176 - protein, 8 aa, synthetic construct
QHSRESLT

SEQ ID NO: 177 - protein, 8 aa, synthetic construct
QHSREHLT

SEQ ID NO: 178 - protein, 8 aa, synthetic construct
QHSRELDT

SEQ ID NO: 179 - protein, 8 aa, synthetic construct
QHSRELLR

SEQ ID NO: 180 - protein, 8 aa, synthetic construct
QHSHELDT

SEQ ID NO: 181 - protein, 8 aa, synthetic construct
QHSHELDR

SEQ ID NO: 182 - protein, 8 aa, synthetic construct
QHSHELDT

SEQ ID NO: 183 - protein, 8 aa, synthetic construct
QHSHELDR

SEQ ID NO: 184 - protein, 119 aa, synthetic construct
QVQLVQSGAEVKKPGASVKVSCKASGYTFTSYVMHWVRQAPGQGLEWMGYINPYNDDTNYNEKFKGRVTMTRDTSTSTVYMELSSLRSEDTAVYYCAREDYYGSRWGKWGQGTLVTVSS

SEQ ID NO: 185 - protein, 119 aa, synthetic construct
QVQLVQSGAEVKKPGASVKVSCKASGYTFTSYVMHWVRQAPGQGLEWMGYINPYNDDTNYNEKFKGRVTMTRDTSTSTVYMELSSLRSEDTAVYYCAREDYYGSRWGTWGQGTLVTVSS

SEQ ID NO: 186 - protein, 110 aa, synthetic construct
DIVLTQSPASLAVSPGQRATITCRASKSVSTSGYSYMHWYQQKPGQPPKLLIYLASNLESGVPARFSGSGSGTDFTLTINPVEANDTANYYCQHSHELLTFGQGTKVEIK

SEQ ID NO: 187 - protein, 110 aa, synthetic construct
DIVLTQSPASLAVSPGQRATITCRASKSVSTSGYSYMHWYQQKPGQPPKLLIYLASNLESGVPARFSGSGSGTDFTLTINPVEANDTANYYCQHSRELDTFGQGTKVEIK

SEQ ID NO: 188 - protein, 110 aa, synthetic construct
DIVLTQSPASLAVSPGQRATITCRASKSVSTSGYSYMHWYQQKPGQPPKLLIYLASNLESGVPARFSGSGSGTDFTLTINPVEANDTANYYCQHSSELLTFGQGTKVEIK

SEQ ID NO: 189 - protein, 110 aa, synthetic construct
DIVLTQSPASLAVSPGQRATITCRASKSVSTSGYSYMHWYQQKPGQPPKLLIYLASNLESGVPARFSGSGSGTDFTLTINPVEANDTANYYCQHSRELLRFGQGTKVEIK

SEQ ID NO: 190 - protein, 110 aa, synthetic construct
DIVLTQSPASLAVSPGQRATITCRASKSVSTSGYSYMHWYQQKPGQPPKLLIYLASNLESGVPARFSGSGSGTDFTLTINPVEANDTANYYCQHSHELDTFGQGTKVEIK

SEQ ID NO: 191 - protein, 110 aa, synthetic construct
DIVLTQSPASLAVSPGQRATITCRASKSVSTSGYSYMHWYQQKPGQPPKLLIYLASNLESGVPARFSGSGSGTDFTLTINPVEANDTANYYCQHSHELDRFGQGTKVEIK

SEQ ID NO: 192 - protein, 13 aa, synthetic construct
SGSSSNIGSNAVN

SEQ ID NO: 193 - protein, 13 aa, synthetic construct
SGSSSNIGNKAVN

SEQ ID NO: 194 - protein, 7 aa, synthetic construct
YDKNRPS

SEQ ID NO: 195 - protein, 11 aa, synthetic construct
AAWDDRLSGYV

SEQ ID NO: 196 - protein, 11 aa, synthetic construct
AAWDRSLSGYV

SEQ ID NO: 197 - protein, 110 aa, synthetic construct
QSVLTQPPSASGTPGQRVTISCSGSSSNIGNNAVNWYQQLPGTAPKLLIYYDKNRPSGVPDRFSGSKSGTSASLAISGLRSEDEADYYCAAWDDRLSGYVFGGGTKLTVL

SEQ ID NO: 198 - protein, 110 aa, synthetic construct
QSVLTQPPSASGTPGQRVTISCSGSSSNIGNNAVNWYQQLPGTAPKLLIYYDKNRPSGVPDRFSGSKSGTSASLAISGLRSEDEADYYCAAWDRSLSGYVFGGGTKLTVL

SEQ ID NO: 199 - protein, 110 aa, synthetic construct
QSVLTQPPSASGTPGQRVTISCSGSSSNIGSNAVNWYQQLPGTAPKLLIYYDSNRPSGVPDRFSGSKSGTSASLAISGLRSEDEADYYCAAWDDSLSGYVFGGGTKLTVL

SEQ ID NO: 200 - protein, 110 aa, synthetic construct
QSVLTQPPSASGTPGQRVTISCSGSSSNIGNKAVNWYQQLPGTAPKLLIYYDSNRPSGVPDRFSGSKSGTSASLAISGLRSEDEADYYCAAWDDSLSGYVFGGGTKLTVL

SEQ ID NO: 201 - DNA, 30 bp, synthetic construct
  source 1..30: mol_type = other DNA
aagcagtggtatcaacgcagagtacgcggg

SEQ ID NO: 202 - DNA, 57 bp, synthetic construct
  source 1..57: mol_type = other DNA
aagcagtggtatcaacgcagagtacttttttttttttttttttttttttttttttvn

SEQ ID NO: 203 - DNA, 23 bp, synthetic construct
  source 1..23: mol_type = other DNA
aagcagtggtatcaacgcagagt

SEQ ID NO: 204 - DNA, 24 bp, synthetic construct
  source 1..24: mol_type = other DNA
caggggccagtggatagaccgatg

SEQ ID NO: 205 - DNA, 24 bp, synthetic construct
  source 1..24: mol_type = other DNA
caggggccagtggatagactgatg

SEQ ID NO: 206 - DNA, 29 bp, synthetic construct
  source 1..29: mol_type = other DNA
ggatggtgggaagatggatacagttggtg

SEQ ID NO: 207 - DNA, 30 bp, synthetic construct
  source 1..30: mol_type = other DNA
ttaacactcattcctgttgaagctcttgac